European Patent Application EP 4 631 972 A1, published October 15, 2025. Title: SITE-SPECIFIC COUPLED PEGYLATED INTERLEUKIN-2 MUTANT WITH RECEPTOR AFFINITY PREFERENCE AND USE THEREOF. Applicant: NANJING NOVOACINE BIOTECHNOLOGY CO., LTD. The sequence listing filed with the application follows.

SEQUENCE LISTING (12 sequences)

SEQ ID NO: 1 - protein, 133 aa, synthetic construct
APTSSSTKKTQLQLEHLLLDLQMILNGINNYKNPKLTRMLTFKFYMPKKATELKHLQCLEEELKPLEEVLNLAQSKNFHLRPRDLISNINVIVLELKGSETTFMCEYADETATIVEFLNRWITFSQSIISTLT

SEQ ID NO: 2 - protein, 133 aa, synthetic construct
  VARIANT 91: note = submitted by C
APTSSSTKKTQLQLEHLLLDLQMILNGINNYKNPKLTRMLTFKFYMPKKATELKHLQCLEEELKPLEEVLNLAQSKNFHLRPRDLISNINXIVLELKGSETTFMCEYADETATIVEFLNRWITFSQSIISTLT

SEQ ID NO: 3 - protein, 133 aa, synthetic construct
  VARIANT 84: note = submitted by C
APTSSSTKKTQLQLEHLLLDLQMILNGINNYKNPKLTRMLTFKFYMPKKATELKHLQCLEEELKPLEEVLNLAQSKNFHLRPRXLISNINVIVLELKGSETTFMCEYADETATIVEFLNRWITFSQSIISTLT

SEQ ID NO: 4 - protein, 133 aa, synthetic construct
  VARIANT 88: note = submitted by C
APTSSSTKKTQLQLEHLLLDLQMILNGINNYKNPKLTRMLTFKFYMPKKATELKHLQCLEEELKPLEEVLNLAQSKNFHLRPRDLISXINVIVLELKGSETTFMCEYADETATIVEFLNRWITFSQSIISTLT

SEQ ID NO: 5 - protein, 133 aa, synthetic construct
  VARIANT 88: note = submitted by R
  VARIANT 33: note = submitted by C
APTSSSTKKTQLQLEHLLLDLQMILNGINNYKXPKLTRMLTFKFYMPKKATELKHLQCLEEELKPLEEVLNLAQSKNFHLRPRDLISXINVIVLELKGSETTFMCEYADETATIVEFLNRWITFSQSIISTLT

SEQ ID NO: 6 - protein, 133 aa, synthetic construct
  VARIANT 75: note = submitted by C
  VARIANT 88: note = submitted by R
APTSSSTKKTQLQLEHLLLDLQMILNGINNYKNPKLTRMLTFKFYMPKKATELKHLQCLEEELKPLEEVLNLAQXKNFHLRPRDLISXINVIVLELKGSETTFMCEYADETATIVEFLNRWITFSQSIISTLT

SEQ ID NO: 7 - protein, 133 aa, synthetic construct
  VARIANT 77: note = submitted by C
  VARIANT 88: note = submitted by R
APTSSSTKKTQLQLEHLLLDLQMILNGINNYKNPKLTRMLTFKFYMPKKATELKHLQCLEEELKPLEEVLNLAQSKXFHLRPRDLISXINVIVLELKGSETTFMCEYADETATIVEFLNRWITFSQSIISTLT

SEQ ID NO: 8 - protein, 133 aa, synthetic construct
  VARIANT 88: note = submitted by R
  VARIANT 109: note = submitted by C
APTSSSTKKTQLQLEHLLLDLQMILNGINNYKNPKLTRMLTFKFYMPKKATELKHLQCLEEELKPLEEVLNLAQSKNFHLRPRDLISXINVIVLELKGSETTFMCEYAXETATIVEFLNRWITFSQSIISTLT

SEQ ID NO: 9 - protein, 133 aa, synthetic construct; identical to SEQ ID NO: 5
  VARIANT 33: note = submitted by p-Acetyl-L-phenylalanine
  VARIANT 88: note = submitted by R

SEQ ID NO: 10 - protein, 133 aa, synthetic construct; identical to SEQ ID NO: 7
  VARIANT 77: note = submitted by p-Acetyl-L-phenylalanine
  VARIANT 88: note = submitted by R

SEQ ID NO: 11 - protein, 133 aa, synthetic construct; identical to SEQ ID NO: 5
  VARIANT 33: note = submitted by N-epsilon-propargyloxycarbonyl-L-lysine
  VARIANT 88: note = submitted by R

SEQ ID NO: 12 - protein, 133 aa, synthetic construct; identical to SEQ ID NO: 7
  VARIANT 77: note = submitted by N-epsilon-propargyloxycarbonyl-L-lysine
  VARIANT 88: note = submitted by R